European Patent Application EP 4 223 776 A1, published August 9, 2023. Title: ANTI-PD-L1 ANTIBODY AND USE THEREOF. Applicant: IMMUNOURCHIN. The sequence listing filed with the application follows.

SEQUENCE LISTING (40 sequences)

SEQ ID NO: 1 - DNA, 37 bp, Artificial Sequence
  hPD-L1-F1
gcgtcggctagcgccaccatgaggatatttgctgtct

SEQ ID NO: 2 - DNA, 33 bp, Artificial Sequence
  hPD-L1-R1
gcgccactcgagttacgtctcctccaaatgtgt

SEQ ID NO: 3 - DNA, 21 bp, Artificial Sequence
  pan IgC-F2
gccccatacaacaaaatcaac

SEQ ID NO: 4 - DNA, 40 bp, Artificial Sequence
  pan IgC-R2
gttgattttgttgtatggggctgcgttcagcaaatgccag

SEQ ID NO: 5 - DNA, 33 bp, Artificial Sequence
  hPD-L1-3-R3
gcgtcgctcgagttaatctccactcaggacttg

SEQ ID NO: 6 - DNA, 36 bp, Artificial Sequence
  hPD-L1-9-R3
gcgtcgctcgagttattctcccaagtgagtcctttc

SEQ ID NO: 7 - DNA, 37 bp, Artificial Sequence
  hPD-1-F4
gcgtcggctagcgccaccatgcagatcccacaggcgc

SEQ ID NO: 8 - DNA, 33 bp, Artificial Sequence
  hPD-1-R4
gcgccactcgagtcagaggggccaagagcagtg

SEQ ID NO: 9 - DNA, 39 bp, Artificial Sequence
  hPD-L2-F5
gcgtcggctagcgccaccatgatcttcctcctgctaatg

SEQ ID NO: 10 - DNA, 33 bp, Artificial Sequence
  hPD-L2-R5
gcgccactcgagtcagatagcactgttcacttc

SEQ ID NO: 11 - protein, 123 aa, Artificial Sequence
  VH of mouse monoclonal antibody #19
EVQLQQSGPELVKPGASVKISCKASGSAFSSSWMNWLKQRPGQGLEWIGRIYPGDGDTNYNGKFKGKATLTADKSSSTAYMQLSSLTSVDSAVYFCARRRANHYGSNWYFDVWGAGTTVTVSS

SEQ ID NO: 12 - protein, 7 aa, Artificial Sequence
  VH-CDR1
GSAFSSS

SEQ ID NO: 13 - protein, 8 aa, Artificial Sequence
  VH-CDR2
IYPGDGDT

SEQ ID NO: 14 - protein, 16 aa, Artificial Sequence
  VH-CDR3
ARRRANHYGSNWYFDV

SEQ ID NO: 15 - protein, 111 aa, Artificial Sequence
  VL of mouse monoclonal antibody #19
NIVLTQSPASLAVSLGQRATISCRASESVDSYGKSFMHWYQQKPGQPPKLLIYLASNLESGVPARFSGSGSRTDFTLTIDPVEADDAATYYCQQNNEDPYTFGGGTKLEIK

SEQ ID NO: 16 - protein, 10 aa, Artificial Sequence
  VL-CDR1
ESVDSYGKSF

SEQ ID NO: 17 - protein, 3 aa, Artificial Sequence
  VL-CDR2
LAS

SEQ ID NO: 18 - protein, 9 aa, Artificial Sequence
  VL-CDR3
QQNNEDPYT

SEQ ID NO: 19 - protein, 290 aa, Artificial Sequence
  PD-L1 protein
MRIFAVFIFMTYWHLLNAFTVTVPKDLYVVEYGSNMTIECKFPVEKQLDLAALIVYWEMEDKNIIQFVHGEEDLKVQHSSYRQRARLLKDQLSLGNAALQITDVKLQDAGVYRCMISYGGADYKRITVKVNAPYNKINQRILVVDPVTSEHELTCQAEGYPKAEVIWTSSDHQVLSGKTTTTNSKREEKLFNVTSTLRINTTTNEIFYCTFRRLDPEENHTAELVIPELPLAHPPNERTHLVILGAILLCLGVALTFIFRLRKGRMMDVKKCGIQDTNSKKQSDTHLEET

SEQ ID NO: 20 - protein, 123 aa, Artificial Sequence
  VH1
EVQLVQSGAEVKKPGSSVKVSCKASGSAFSSSWMNWLRQAPGQGLEWMGRIYPGDGDTNYNQKFQGRVTLTADKSTSTAYMELSSLRSVDTAVYFCARRRANHYGSNWYFDVWGQGTTVTVSS

SEQ ID NO: 21 - protein, 123 aa, Artificial Sequence
  VH2
QVQLVQSGAEVKKPGASVKVSCKASGSAFSSSWMNWLRQAPGQGLEWIGRIYPGDGDTNYNQKFQGRVTLTADSSISTAYMELSRLRSVDTVVYFCARRRANHYGSNWYFDVWGQGTTVTVSS

SEQ ID NO: 22 - protein, 123 aa, Artificial Sequence
  VH3
EVQLVQSGAEVKKPGASVKVSCKASGSAFSSSWMNWLRQAPGQGLEWMGRIYPGDGDTNYNQKFQGRVTLTADKSISTAYMELSRLRSVDTAVYFCARRRANHYGSNWYFDVWGQGTTVTVSS

SEQ ID NO: 23 - protein, 123 aa, Artificial Sequence
  VH4
EVQLVQSGAEVKKPGSSVKVSCKASGSAFSSSWMNWLRQRPGQGLEWIGRIYPGDGDTNYNGKFKGRVTLTADKSSSTAYMELSSLRSVDTAVYFCARRRANHYGSNWYFDVWGAGTTVTVSS

SEQ ID NO: 24 - protein, 123 aa, Artificial Sequence
  VH5
EVQLVQSGAEVKKPGASVKVSCKASGSAFSSSWMNWLRQRPGQGLEWIGRIYPGDGDTNYNGKFKGRVTLTADKSISTAYMELSRLRSVDTAVYFCARRRANHYGSNWYFDVWGAGTTVTVSS

SEQ ID NO: 25 - protein, 123 aa, Artificial Sequence
  VH6
EVQLQQSGAEVKKPGSSVKVSCKASGSAFSSSWMNWLKQRPGQGLEWIGRIYPGDGDTNYNGKFKGRVTLTADKSSSTAYMQLSSLRSEDTAVYFCARRRANHYGSNWYFDVWGAGTTVTVSS

SEQ ID NO: 26 - protein, 111 aa, Artificial Sequence
  VL1
NIVLTQSPATLSLSPGERATLSCRASESVDSYGKSFMHWYQQKPGQPPKLLIYLASNLETGIPARFSGSGSRTDFTLTISSLEPEDFAVYYCQQNNEDPYTFGGGTKLEIK

SEQ ID NO: 27 - protein, 111 aa, Artificial Sequence
  VL2
NIVLTQSPSSLSASVGDRVTITCRASESVDSYGKSFMHWYQQKPGQPPKLLIYLASNLESGVPSRFSGSGSRTDFTLTISSLQPEDFATYYCQQNNEDPYTFGGGTKLEIK

SEQ ID NO: 28 - protein, 111 aa, Artificial Sequence
  VL3
NIVLTQSPATLSLSPGERATLSCRASESVDSYGKSFMHWYQQKPGQPPKLLIYLASNLETGIPARFSGSGSRTDFTLTIDSLEPEDFAVYYCQQNNEDPYTFGGGTKLEIK

SEQ ID NO: 29 - protein, 111 aa, Artificial Sequence
  VL4
NIVLTQSPASLSASVGDRVTISCRASESVDSYGKSFMHWYQQKPGQPPKLLIYLASNLESGVPARFSGSGSRTDFTLTISSLQPEDFATYYCQQNNEDPYTFGGGTKLEIK

SEQ ID NO: 30 - protein, 111 aa, Artificial Sequence
  VL5
NIVLTQSPASLSASVGDRVTISCRASESVDSYGKSFMHWYQQKPGQPPKLLIYLASNLESGVPARFSGSGSRTDFTLTIDSLQPEDFATYYCQQNNEDPYTFGGGTKLEIK

SEQ ID NO: 31 - DNA, 873 bp, Artificial Sequence
  Membrane PDL1
atgaggatatttgctgtctttatattcatgacctactggcatttgctgaacgcatttactgtcacggttcccaaggacctatatgtggtagagtatggtagcaatatgacaattgaatgcaaattcccagtagaaaaacaattagacctggctgcactaattgtctattgggaaatggaggataagaacattattcaatttgtgcatggagaggaagacctgaaggttcagcatagtagctacagacagagggcccggctgttgaaggaccagctctccctgggaaatgctgcacttcagatcacagatgtgaaattgcaggatgcaggggtgtaccgctgcatgatcagctatggtggtgccgactacaagcgaattactgtgaaagtcaatgccccatacaacaaaatcaaccaaagaattttggttgtggatccagtcacctctgaacatgaactgacatgtcaggctgagggctaccccaaggccgaagtcatctggacaagcagtgaccatcaagtcctgagtggtaagaccaccaccaccaattccaagagagaggagaagcttttcaatgtgaccagcacactgagaatcaacacaacaactaatgagattttctactgcacttttaggagattagatcctgaggaaaaccatacagctgaattggtcatcccagaactacctctggcacatcctccaaatgaaaggactcacttggtaattctgggagccatcttattatgccttggtgtagcactgacattcatcttccgtttaagaaaagggagaatgatggatgtgaaaaaatgtggcatccaagatacaaactcaaagaagcaaagtgatacacatttggaggagacgtaa

SEQ ID NO: 32 - protein, 290 aa, Artificial Sequence; identical to SEQ ID NO: 19
  Membrane PDL1

SEQ ID NO: 33 - DNA, 873 bp, Artificial Sequence
  PDL1-1 splicing variant
atgaggatatttgctgtctttatattcatgacctactggcatttgctgaacgcatttactgtcacggttcccaaggacctatatgtggtagagtatggtagcaatatgacaattgaatgcaaattcccagtagaaaaacaattagacctggctgcactaattgtctattgggaaatggaggataagaacattattcaatttgtgcatggagaggaagacctgaaggttcagcatagtagctacagacagagggcccggctgttgaaggaccagctctccctgggaaatgctgcacttcagatcacagatgtgaaattgcaggatgcaggggtgtaccgctgcatgatcagctatggtggtgccgactacaagcgaattactgtgaaagtcaatgccccatacaacaaaatcaaccaaagaattttggttgtggatccagtcacctctgaacatgaactgacatgtcaggctgagggctaccccaaggccgaagtcatctggacaagcagtgaccatcaagtcctgagtggtaagaccaccaccaccaattccaagagagaggagaagcttttcaatgtgaccagcacactgagaatcaacacaacaactaatgagattttctactgcacttttaggagattagatcctgaggaaaaccatacagctgaattggtcatcccagaactacctctggcacatcccccaaatgaaaggactcacttggtaattctgggagccatcttattatgccttggtgtagcactgacattcatcttccgtttaagaaaagggagaatgatggatgtgaaaaaatgtggcatccaagatacaaactcaaagaagcaaagtgatacacatttggaggagacgtaa

SEQ ID NO: 34 - protein, 270 aa, Artificial Sequence
  PDL1-1 splicing variant
MRIFAVFIFMTYWHLLNAFTVTVPKDLYVVEYGSNMTIECKFPVEKQLDLAALIVYWEMEDKNIIQFVHGEEDLKVQHSSYRQRARLLKDQLSLGNAALQITDVKLQDAGVYRCMISYGGADYKRITVKVNAPYNKINQRILVVDPVTSEHELTCQAEGYPKAEVIWTSSDHQVLSGKTTTTNSKREEKLFNVTSTLRINTTTNEIFYCTFRRLDPEENHTAELVIPELPLAHPPNERTHLVILGAILLCLGVALTFIFRLRKDTHLEET

SEQ ID NO: 35 - DNA, 873 bp, Artificial Sequence; identical to SEQ ID NO: 31
  PDL1-3 splicing variant

SEQ ID NO: 36 - protein, 178 aa, Artificial Sequence
  PDL1-3 splicing variant
MRIFAVFIFMTYWHLLNAFTVTVPKDLYVVEYGSNMTIECKFPVEKQLDLAALIVYWEMEDKNIIQFVHGEEDLKVQHSSYRQRARLLKDQLSLGNAALQITDVKLQDAGVYRCMISYGGADYKRITVKVNAPYNKINQRILVVDPVTSEHELTCQAEGYPKAEVIWTSSDHQVLSGD

SEQ ID NO: 37 - DNA, 873 bp, Artificial Sequence; identical to SEQ ID NO: 31
  PDL1-9 splicing variant

SEQ ID NO: 38 - protein, 243 aa, Artificial Sequence
  PDL1-9 splicing variant
MRIFAVFIFMTYWHLLNAFTVTVPKDLYVVEYGSNMTIECKFPVEKQLDLAALIVYWEMEDKNIIQFVHGEEDLKVQHSSYRQRARLLKDQLSLGNAALQITDVKLQDAGVYRCMISYGGADYKRITVKVNAPYNKINQRILVVDPVTSEHELTCQAEGYPKAEVIWTSSDHQVLSGKTTTTNSKREEKLFNVTSTLRINTTTNEIFYCTFRRLDPEENHTAELVIPELPLAHPPNERTHLGE

SEQ ID NO: 39 - DNA, 873 bp, Artificial Sequence; identical to SEQ ID NO: 31
  PDL1-12 splicing variant

SEQ ID NO: 40 - protein, 178 aa, Artificial Sequence
  PDL1-12 splicing variant
MRIFAVFIFMTYWHLLNAFTVTVPKDLYVVEYGSNMTIECKFPVEKQLDLAALIVYWEMEDKNIIQFVHGEEDLKVQHSSYRQRARLLKDQLPLGNAALQITDVKLQDAGVYRCMISYGGADYKRITVKVNAPYNKINQRILVVDPVTSEHELTCQAEGYPKAEVIWTSSDHQVLSGD